European Patent Specification EP 3 997 229 B1, published June 3, 2026. Title: TARGETED RNA EDITING BY LEVERAGING ENDOGENOUS ADAR USING ENGINEERED RNAS. Applicant: Peking University. The sequence listing filed with the application follows.

SEQUENCE LISTING (51 sequences)

SEQ ID NO: 1 - DNA, 122 bp, Artificial Sequence
  Synthesized sequence
aagattgtgtgtggatcgatgatgacttccatatatacattccttggaaagctgaacaaaatgagtgaaaactctataccgtcattctcgtcgaactgaggtccagcacattactccaacag

SEQ ID NO: 2 - DNA, 116 bp, Artificial Sequence
  Synthesized sequence
gagtgagatcttggaccaatgatgacttccatacatgcattccttggaaagctgaacaaaatgagtgggaactctgtactatcatcttagttgaactgaggtccaccgggggctaa

SEQ ID NO: 3 - DNA, 508 bp, Artificial Sequence
  Synthesized sequence
cgttacataacttacggtaaatggcccgcctggctgaccgcccaacgacccccgcccattgacgtcaataatgacgtatgttcccatagtaacgccaatagggactttccattgacgtcaatgggtggagtatttacggtaaactgcccacttggcagtacatcaagtgtatcatatgccaagtacgccccctattgacgtcaatgacggtaaatggcccgcctggcattatgcccagtacatgaccttatgggactttcctacttggcagtacatctacgtattagtcatcgctattaccatggtgatgcggttttggcagtacatcaatgggcgtggatagcggtttgactcacggggatttccaagtctccaccccattgacgtcaatgggagtttgttttggcaccaaaatcaacgggactttccaaaatgtcgtaacaactccgccccattgacgcaaatgggcggtaggcgtgtacggtgggaggtctatataagcagagct

SEQ ID NO: 4 - RNA, 111 nt, Artificial Sequence
  Synthesized sequence
gggagcagccucuggcauucugggagcuucaucuggaccugggucuucagugaaccauuguucaauaucguccggggacagcaucaaaucauccauugcuugggacggcaa

SEQ ID NO: 5 - RNA, 111 nt, Artificial Sequence
  Synthesized sequence
gacgcccaccgugugguugcuguccaggacggucccggccugcgacacuucggcccagagcugcuccucaucugcggggcgggggggggccgucgccgcguggggucguug

SEQ ID NO: 6 - RNA, 111 nt, Artificial Sequence
  Synthesized sequence
cauauuacagaauaccuugauagcauccaauuugcauccuugguuagggucaacccaguauucuccacucuugaguucaggauggcagaauuucaggucucugcaguuucu

SEQ ID NO: 7 - RNA, 111 nt, Artificial Sequence
  Synthesized sequence
gugaagauaagccaguccucuaguaacagaaugagcaagacggcaagagcuuacccagucacuuguguggagacuuaaauacuugcauaaagauccauugggauaguacuc

SEQ ID NO: 8 - RNA, 111 nt, Artificial Sequence
  Synthesized sequence
gugaacgucaaacugucggaccaauauggcagaaucuucucucaucucaacuuuccauauccguaucauggaaucauagcauccuguaacuacuagcucucuuacagcugg

SEQ ID NO: 9 - RNA, 111 nt, Artificial Sequence
  Synthesized sequence
gccaaugaucucgugaguuaucucagcagugugagccaucagggugaugacaucccaggcgaucguguggccuccaggagcccagagcaggaaguugaggagaaggugccu

SEQ ID NO: 10 - RNA, 111 nt, Artificial Sequence
  Synthesized sequence
caagacggugaaccacuccauggucuucuugucggcuuucugcacuguguacccccagagcuccguguugccgacauccugggguggcuuccacuccagagccacauuaag

SEQ ID NO: 11 - RNA, 111 nt, Artificial Sequence
  Synthesized sequence
aggauucucuuuugaaguauugcucccccaguggauuggguggcuccauucacuccaaugcugagcacuuccacagaguggguuaaagcggcuccgaacacgaaacgugua

SEQ ID NO: 12 - DNA, 31 bp, Artificial Sequence
  Synthesized sequence
tataactagtatggtgagcaagggcgaggag

SEQ ID NO: 13 - DNA, 41 bp, Artificial Sequence
  Synthesized sequence
tatacgtctcatctacagattcttccggcgtgtataccttc

SEQ ID NO: 14 - DNA, 53 bp, Artificial Sequence
  Synthesized sequence
tatacgtctcatagagatccccggtcgccaccgtgagcaagggcgaggagctg

SEQ ID NO: 15 - DNA, 51 bp, Artificial Sequence
  Synthesized sequence
uaaaccgagggaucauaggggacugaauccaccauucuucucccaaucccu

SEQ ID NO: 16 - DNA, 151 bp, Artificial Sequence
  Synthesized sequence
acuacaguugcuccgauauuuaggcuacgucaauaggcacuaacuuauuggcgcuggugaacggacuuccucucgaguaccagaagaugacuacaaaacuccuuuccauugcgaguaucggagucuggcucaguuuggccagggaggcacu

SEQ ID NO: 17 - DNA, 51 bp, Artificial Sequence
  Synthesized sequence
gcccttgctcactggcagagccctccagcatcgcgagcaggcgctgcctcc

SEQ ID NO: 18 - DNA, 151 bp, Artificial Sequence; identical to SEQ ID NO: 16
  Synthesized sequence

SEQ ID NO: 19 - DNA, 116 bp, Artificial Sequence; identical to SEQ ID NO: 2
  Synthesized sequence

SEQ ID NO: 20 - DNA, 122 bp, Artificial Sequence; identical to SEQ ID NO: 1
  Synthesized sequence

SEQ ID NO: 21 - DNA, 708 bp, Artificial Sequence
  Synthesized sequence
atggtgagcaagggcgaggaggataacatggccatcatcaaggagttcatgcgcttcaaggtgcacatggagggctccgtgaacggccacgagttcgagatcgagggcgagggcgagggccgcccctacgagggcacccagaccgccaagctgaaggtgaccaagggtggccccctgcccttcgcctgggacatcctgtcccctcagttcatgtacggctccaaggcctacgtgaagcaccccgccgacatccccgactacttgaagctgtccttccccgagggcttcaagtgggagcgcgtgatgaacttcgaggacggcggcgtggtgaccgtgacccaggactcctccctgcaggacggcgagttcatctacaaggtgaagctgcgcggcaccaacttcccctccgacggccccgtaatgcagaagaagaccatgggctgggaggcctcctccgagcggatgtaccccgaggacggcgccctgaagggcgagatcaagcagaggctgaagctgaaggacggcggccactacgacgctgaggtcaagaccacctacaaggccaagaagcccgtgcagctgcccggcgcctacaacgtcaacatcaagttggacatcacctcccacaacgaggactacaccatcgtggaacagtacgaacgcgccgagggccgccactccaccggcggcatggacgagctgtacaag

SEQ ID NO: 22 - DNA, 99 bp, Artificial Sequence
  Synthesized sequence
ctgcagggcggaggaggcagcggcggaggaggcagcggcggaggaggcagcagaaggtatacacgccggaagaatctgtagagatccccggtcgccacc

SEQ ID NO: 23 - DNA, 717 bp, Artificial Sequence
  Synthesized sequence
gtgagcaagggcgaggagctgttcaccggggtggtgcccatcctggtcgagctggacggcgacgtaaacggccacaagttcagcgtgtccggcgagggcgagggcgatgccacctacggcaagctgaccctgaagttcatctgcaccaccggcaagctgcccgtgccctggcccaccctcgtgaccaccctgacctacggcgtgcagtgcttcagccgctaccccgaccacatgaagcagcacgacttcttcaagtccgccatgcccgaaggctacgtccaggagcgcaccatcttcttcaaggacgacggcaactacaagacccgcgccgaggtgaagttcgagggcgacaccctggtgaaccgcatcgagctgaagggcatcgacttcaaggaggacggcaacatcctggggcacaagctggagtacaactacaacagccacaacgtctatatcatggccgacaagcagaagaacggcatcaaggtgaacttcaagatccgccacaacatcgaggacggcagcgtgcagctcgccgaccactaccagcagaacacccccatcggcgacggccccgtgctgctgcccgacaaccactacctgagcacccagtccgccctgagcaaagaccccaacgagaagcgcgatcacatggtcctgctggagttcgtgaccgccgccgggatcactctcggcatggacgagctgtacaagtaa

SEQ ID NO: 24 - DNA, 51 bp, Artificial Sequence
  Synthesized sequence
ctgcagggcggaggaggcagcgcctgctcgcgatgctagagggctctgcca

SEQ ID NO: 25 - RNA, 21 nt, Artificial Sequence
  Synthesized sequence
aaccaugccgacugauggcag

SEQ ID NO: 26 - RNA, 26 nt, Artificial Sequence
  Synthesized sequence
cugccaucagucggcguggacuguag

SEQ ID NO: 27 - RNA, 71 nt, Artificial Sequence
  Synthesized sequence
acagcuccucgcccuugcucacuggcagagcccuccagcaucgcgagcaggcgcugccuccuccgccgcug

SEQ ID NO: 28 - RNA, 121 nt, Artificial Sequence
  Synthesized sequence
cacacacaaacacacacaacacaacacagcuccucgcccuugcucacuggcagagcccuccagcaucgcgagcaggcgcugccuccuccgccgcugcaacacacaaaaccaccacaccaac

SEQ ID NO: 29 - RNA, 171 nt, Artificial Sequence
  Synthesized sequence
accacacacacaaccaccacacacacacacacaaacacacacaacacaacacagcuccucgcccuugcucacuggcagagcccuccagcaucgcgagcaggcgcugccuccuccgccgcugcaacacacaaaaccaccacaccaaccccaacaaccacacacccacacaac

SEQ ID NO: 30 - RNA, 111 nt, Artificial Sequence
  Synthesized sequence
gaugggcaccaccccggugaacagcuccucgcccuugcucacuggcagagcccuccagcaucgcgagcaggcgcugccuccuccgccgcugccuccuccgccgcugccucc

SEQ ID NO: 31 - RNA, 161 nt, Artificial Sequence
  Synthesized sequence
cacacacaaacacacacaacacaacgaugggcaccaccccggugaacagcuccucgcccuugcucacuggcagagcccuccagcaucgcgagcaggcgcugccuccuccgccgcugccuccuccgccgcugccucccaacacacaaaaccaccacaccaac

SEQ ID NO: 32 - RNA, 211 nt, Artificial Sequence
  Synthesized sequence
accacacacacaaccaccacacacacacacacaaacacacacaacacaacgaugggcaccaccccggugaacagcuccucgcccuugcucacuggcagagcccuccagcaucgcgagcaggcgcugccuccuccgccgcugccuccuccgccgcugccucccaacacacaaaaccaccacaccaaccccaacaaccacacacccacacaac

SEQ ID NO: 33 - RNA, 123 nt, Artificial Sequence
  Synthesized sequence
uugccauguguauguggggagacggucggguccagauauucguaucugucgaguagagugugggcuccccacauacucugaugauccagagacgauauuacgucucaggaucauucauggcaa

SEQ ID NO: 34 - RNA, 71 nt, Artificial Sequence; identical to SEQ ID NO: 27
  Synthesized sequence

SEQ ID NO: 35 - RNA, 71 nt, Artificial Sequence
  Synthesized sequence
uuucagcuauaccugcccgguauaaagggacguucacaccgcgauguucucugcuggggaauugcgcgaua

SEQ ID NO: 36 - RNA, 111 nt, Artificial Sequence; identical to SEQ ID NO: 30
  Synthesized sequence

SEQ ID NO: 37 - RNA, 111 nt, Artificial Sequence
  Synthesized sequence
uaccgcuacagccacgcugauuucagcuauaccugcccgguauaaagggacguucacaccgcgauguucucugcuggggaauugcgcgauauucaggauuaaaagaagugc

SEQ ID NO: 38 - RNA, 151 nt, Artificial Sequence
  Synthesized sequence
acuacaguugcuccgauauuuaggcuacgucaauaggcacuaacuuauuggcgcuggugaacggacuuccucucgaguaccagaagaugacuacaaaacuccuuuccauugcgaguaucggagucuggcucaguuuggccagggaggcacu

SEQ ID NO: 39 - RNA, 31 nt, Artificial Sequence
  Synthesized sequence
acuggcagagcccuccagcaucgcgagcagg

SEQ ID NO: 40 - RNA, 51 nt, Artificial Sequence
  Synthesized sequence
gcccuugcucacuggcagagcccuccagcaucgcgagcaggcgcugccucc

SEQ ID NO: 41 - RNA, 71 nt, Artificial Sequence
  Synthesized sequence
acagcuccucgcccuugcucacuggcagagcccuccagcaucgcgagcaggcgcugccuccuccgcccugc

SEQ ID NO: 42 - RNA, 91 nt, Artificial Sequence
  Synthesized sequence
accccggugaacagcuccucgcccuugcucacuggcagagcccuccagcaucgcgagcaggcgcugccuccuccgcccugcagcuuguaca

SEQ ID NO: 43 - RNA, 111 nt, Artificial Sequence
  Synthesized sequence
gaugggcaccaccccggugaacagcuccucgcccuugcucacuggcagagcccuccagcaucgcgagcaggcgcugccuccuccgcccugcagcuuguacagcucguccau

SEQ ID NO: 44 - RNA, 131 nt, Artificial Sequence
  Synthesized sequence
gcucgaccaggaugggcaccaccccggugaacagcuccucgcccuugcucacuggcagagcccuccagcaucgcgagcaggcgcugccuccuccgcccugcagcuuguacagcucguccaugccgccggug

SEQ ID NO: 45 - RNA, 151 nt, Artificial Sequence
  Synthesized sequence
ucgccguccagcucgaccaggaugggcaccaccccggugaacagcuccucgcccuugcucacuggcagagcccuccagcaucgcgagcaggcgcugccuccuccgcccugcagcuuguacagcucguccaugccgccgguggaguggcggc

SEQ ID NO: 46 - RNA, 111 nt, Artificial Sequence; identical to SEQ ID NO: 30
  Synthesized sequence

SEQ ID NO: 47 - RNA, 111 nt, Artificial Sequence; identical to SEQ ID NO: 37
  Synthesized sequence

SEQ ID NO: 48 - RNA, 111 nt, Artificial Sequence; identical to SEQ ID NO: 30
  Synthesized sequence

SEQ ID NO: 49 - RNA, 111 nt, Artificial Sequence; identical to SEQ ID NO: 37
  Synthesized sequence

SEQ ID NO: 50 - RNA, 74 nt, Artificial Sequence
  Synthesized sequence
gcagcggcggaggaggcagcgccugcucgcgaugcuagagggcucugccagugagcaagggcgaggagcuguuc

SEQ ID NO: 51 - RNA, 87 nt, Artificial Sequence
  Synthesized sequence
gagcuguacaagcugcagggcggaggaggcagcgccugcucgcgaugcuagagggcucugccagugagcaagggcgaggagcuguuc